European Patent Application EP 4 631 963 A1, published October 15, 2025. Title: Peptide for cartilage regeneration and uses thereof. Applicant: CAREGEN CO., LTD. The sequence listing filed with the application follows.

SEQUENCE LISTING (13 sequences)

SEQ ID NO: 1 - protein, 6 aa, synthetic construct
HHEERY

SEQ ID NO: 2 - DNA, 23 bp, synthetic construct
  source 1..23: mol_type = other DNA
ctatctggacgaagcagctggca

SEQ ID NO: 3 - DNA, 22 bp, synthetic construct
  source 1..22: mol_type = other DNA
atgggtgcaatgtcaatgatgg

SEQ ID NO: 4 - DNA, 20 bp, synthetic construct
  source 1..20: mol_type = other DNA
aactcagggcaggaggatgt

SEQ ID NO: 5 - DNA, 20 bp, synthetic construct
  source 1..20: mol_type = other DNA
tgtccttttggtcgtcgttc

SEQ ID NO: 6 - DNA, 20 bp, synthetic construct
  source 1..20: mol_type = other DNA
ccagcccgaacttgtaaaga

SEQ ID NO: 7 - DNA, 20 bp, synthetic construct
  source 1..20: mol_type = other DNA
tggacgcacaaccatcatac

SEQ ID NO: 8 - DNA, 20 bp, synthetic construct
  source 1..20: mol_type = other DNA
gcaggctatgagcagtgtga

SEQ ID NO: 9 - DNA, 20 bp, synthetic construct
  source 1..20: mol_type = other DNA
gcatacctcggaagcagaag

SEQ ID NO: 10 - DNA, 20 bp, synthetic construct
  source 1..20: mol_type = other DNA
accacagtccatgccatcac

SEQ ID NO: 11 - DNA, 20 bp, synthetic construct
  source 1..20: mol_type = other DNA
tccaccaccctgttgctgta

SEQ ID NO: 12 - DNA, 20 bp, synthetic construct
  source 1..20: mol_type = other DNA
gcggaggaagtcggtgaaga

SEQ ID NO: 13 - DNA, 20 bp, synthetic construct
  source 1..20: mol_type = other DNA
ccctctcgcttcaggtcagc